European Patent Specification EP 3 727 461 B1, published July 9, 2025. Title: BICYCLIC PEPTIDE LIGANDS SPECIFIC FOR EphA2. Applicant: BicycleTx Limited. The sequence listing filed with the application follows.

SEQUENCE LISTING (98 sequences)

SEQ ID NO: 1 - protein, 15 aa, Artificial
  Synthetic Peptide
  Xaa (2)..(2): X represents HyP
  Xaa (12)..(12): Xaa represents D-Asp
  Xaa (14)..(14): Xaa represents HArg
CXLVNPLCLHPXWXC

SEQ ID NO: 2 - protein, 20 aa, Artificial
  Synthetic Peptide
  Xaa (1)..(1): Xaa represents Beta-Ala
  Xaa (2)..(2): Xaa represents Sar10
  Xaa (4)..(4): Xaa represents HArg
  Xaa (7)..(7): Xaa represents HyP
  Xaa (17)..(17): Xaa represents D-Asp
  Xaa (19)..(19): Xaa represents HArg
XXAXDCXLVNPLCLHPXWXC

SEQ ID NO: 3 - protein, 15 aa, Artificial
  Synthetic peptide
ACMNDWWCAMGWKCA

SEQ ID NO: 4 - protein, 15 aa, Artificial
  Synthetic peptide
ACVPDRRCAYMNVCA

SEQ ID NO: 5 - protein, 15 aa, Artificial
  Synthetic peptide
ACVVDGRCAYMNVCA

SEQ ID NO: 6 - protein, 15 aa, Artificial
  Synthetic peptide
ACVVDSRCAYMNVCA

SEQ ID NO: 7 - protein, 15 aa, Artificial
  Synthetic peptide
ACVPDSRCAYMNVCA

SEQ ID NO: 8 - protein, 15 aa, Artificial
  Synthetic peptide
ACYVGKECAIRNVCA

SEQ ID NO: 9 - protein, 15 aa, Artificial
  Synthetic peptide
ACYVGKECAYMNVCA

SEQ ID NO: 10 - protein, 18 aa, Artificial
  Synthetic peptide
ARDCPLVNPLCLHPGWTC

SEQ ID NO: 11 - protein, 18 aa, Artificial
  Synthetic peptide
  Xaa (2)..(2): Xaa is HArg
AXDCPLVNPLCLHPGWTC

SEQ ID NO: 12 - protein, 18 aa, Artificial
  Synthetic peptide
CPLVNPLCLHPGWTCLHG

SEQ ID NO: 13 - protein, 18 aa, Artificial
  Synthetic peptide
  Xaa (17)..(17): Xaa is D-His
CPLVNPLCLHPGWTCLXG

SEQ ID NO: 14 - protein, 18 aa, Artificial
  Synthetic peptide
CPLVNPLCLHPGWSCRGQ

SEQ ID NO: 15 - protein, 18 aa, Artificial
  Synthetic peptide
  Xaa (16)..(16): Xaa is HArg
CPLVNPLCLHPGWSCXGQ

SEQ ID NO: 16 - protein, 14 aa, Artificial
  Synthetic peptide
ACVPDRRCAYMNVC

SEQ ID NO: 17 - protein, 17 aa, Artificial
  Synthetic peptide
DLRCGGDPRCAYMNVCA

SEQ ID NO: 18 - protein, 17 aa, Artificial
  Synthetic peptide
SRPCVIDSRCAYMNVCA

SEQ ID NO: 19 - protein, 17 aa, Artificial
  Synthetic peptide
ESRCSPDARCAYMNVCA

SEQ ID NO: 20 - protein, 17 aa, Artificial
  Synthetic peptide
HSGCRPDPRCAYMNVCA

SEQ ID NO: 21 - protein, 17 aa, Artificial
  Synthetic peptide
GSGCKPDSRCAYMNVCA

SEQ ID NO: 22 - protein, 17 aa, Artificial
  Synthetic peptide
ETVCLPDSRCAYMNVCA

SEQ ID NO: 23 - protein, 17 aa, Artificial
  Synthetic peptide
GQVCIVDARCAYMNVCA

SEQ ID NO: 24 - protein, 17 aa, Artificial
  Synthetic peptide
ACVPDRRCAFENVCVDH

SEQ ID NO: 25 - protein, 17 aa, Artificial
  Synthetic peptide
ACVPDRRCAFMNVCEDR

SEQ ID NO: 26 - protein, 17 aa, Artificial
  Synthetic peptide
ACVPDRRCAFQDVCDHE

SEQ ID NO: 27 - protein, 17 aa, Artificial
  Synthetic peptide
ACVPDRRCAFRDVCLTG

SEQ ID NO: 28 - protein, 15 aa, Artificial
  Synthetic peptide
ACQPSNHCAFMNYCA

SEQ ID NO: 29 - protein, 15 aa, Artificial
  Synthetic peptide
ACSPTPACAVQNLCA

SEQ ID NO: 30 - protein, 14 aa, Artificial
  Synthetic peptide
ACTSCWAYPDSFCA

SEQ ID NO: 31 - protein, 17 aa, Artificial
  Synthetic peptide
ACTKPTGFCAYPDTICA

SEQ ID NO: 32 - protein, 17 aa, Artificial
  Synthetic peptide
ACRGEWGYCAYPDTICA

SEQ ID NO: 33 - protein, 17 aa, Artificial
  Synthetic peptide
ACRNWGMYCAYPDTICA

SEQ ID NO: 34 - protein, 17 aa, Artificial
  Synthetic peptide
ACPDWGKYCAYPDTICA

SEQ ID NO: 35 - protein, 17 aa, Artificial
  Synthetic peptide
ACRVYGPYCAYPDTICA

SEQ ID NO: 36 - protein, 14 aa, Artificial
  Synthetic peptide
ACSSCWAYPDSVCA

SEQ ID NO: 37 - protein, 14 aa, Artificial
  Synthetic peptide
ACQSCWAYPDTYCA

SEQ ID NO: 38 - protein, 15 aa, Artificial
  Synthetic peptide
ACGFMGLEPCETFCA

SEQ ID NO: 39 - protein, 15 aa, Artificial
  Synthetic peptide
ACGFMGLVPCEVHCA

SEQ ID NO: 40 - protein, 15 aa, Artificial
  Synthetic peptide
ACGFMGLEPCEMVCA

SEQ ID NO: 41 - protein, 15 aa, Artificial
  Synthetic peptide
ACGFMGLEPCVTYCA

SEQ ID NO: 42 - protein, 15 aa, Artificial
  Synthetic peptide
ACGFMGLEPCELVCA

SEQ ID NO: 43 - protein, 15 aa, Artificial
  Synthetic peptide
ACGFMGLVPCNVFCA

SEQ ID NO: 44 - protein, 15 aa, Artificial
  Synthetic peptide
ACGFMGLEPCELFCA

SEQ ID NO: 45 - protein, 17 aa, Artificial
  Synthetic peptide
ACGFMGLEPCELFCMPK

SEQ ID NO: 46 - protein, 15 aa, Artificial
  Synthetic peptide
ACGFMGLEPCELYCA

SEQ ID NO: 47 - protein, 17 aa, Artificial
  Synthetic peptide
ACGFMGLEPCELYCAHT

SEQ ID NO: 48 - protein, 15 aa, Artificial
  Synthetic peptide
ACGFMGLEPCEMYCA

SEQ ID NO: 49 - protein, 17 aa, Artificial
  Synthetic peptide
ACGFMGLVPCELYCADN

SEQ ID NO: 50 - protein, 17 aa, Artificial
  Synthetic peptide
ACPLVNPLCLTSGWKCA

SEQ ID NO: 51 - protein, 17 aa, Artificial
  Synthetic peptide
ACPMVNPLCLHPGWICA

SEQ ID NO: 52 - protein, 17 aa, Artificial
  Synthetic peptide
ACPLVNPLCLHPGWICA

SEQ ID NO: 53 - protein, 17 aa, Artificial
  Synthetic peptide
ACPLVNPLCLHPGWRCA

SEQ ID NO: 54 - protein, 17 aa, Artificial
  Synthetic peptide
ACPLVNPLCNLPGWTCA

SEQ ID NO: 55 - protein, 17 aa, Artificial
  Synthetic peptide
ACPLVNPLCLVPGWSCA

SEQ ID NO: 56 - protein, 17 aa, Artificial
  Synthetic peptide
ACPLVNPLCLLDGWTCA

SEQ ID NO: 57 - protein, 17 aa, Artificial
  Synthetic peptide
ACPLVNPLCLMPGWGCA

SEQ ID NO: 58 - protein, 17 aa, Artificial
  Synthetic peptide
ACPLVNPLCMIGNWTCA

SEQ ID NO: 59 - protein, 17 aa, Artificial
  Synthetic peptide
ACPLVNPLCLMTGWSCA

SEQ ID NO: 60 - protein, 17 aa, Artificial
  Synthetic peptide
ACPLVNPLCMMGGWKCA

SEQ ID NO: 61 - protein, 17 aa, Artificial
  Synthetic peptide
ACPLVNPLCLYGSWKCA

SEQ ID NO: 62 - protein, 17 aa, Artificial
  Synthetic peptide
ACPLVNPLCLHPGWTCA

SEQ ID NO: 63 - protein, 19 aa, Artificial
  Synthetic peptide
ARDCPLVNPLCLHPGWTCA

SEQ ID NO: 64 - protein, 19 aa, Artificial
  Synthetic peptide
RPACPLVNPLCLHPGWTCA

SEQ ID NO: 65 - protein, 19 aa, Artificial
  Synthetic peptide
RPPCPLVNPLCLHPGWTCA

SEQ ID NO: 66 - protein, 19 aa, Artificial
  Synthetic peptide
KHSCPLVNPLCLHPGWTCA

SEQ ID NO: 67 - protein, 19 aa, Artificial
  Synthetic peptide
ACPLVNPLCLHPGWTCLHG

SEQ ID NO: 68 - protein, 19 aa, Artificial
  Synthetic peptide
  Xaa (18)..(18): Xaa is D-His
ACPLVNPLCLHPGWTCLXG

SEQ ID NO: 69 - protein, 19 aa, Artificial
  Synthetic peptide
  Xaa (14)..(14): Xaa is 2Nal
ACPLVNPLCLHPGXTCLHG

SEQ ID NO: 70 - protein, 19 aa, Artificial
  Synthetic peptide
RHDCPLVNPLCLLPGWTCA

SEQ ID NO: 71 - protein, 19 aa, Artificial
  Synthetic peptide
TPRCPLVNPLCLMPGWTCA

SEQ ID NO: 72 - protein, 17 aa, Artificial
  Synthetic peptide
ACPLVNPLCLAPGWTCA

SEQ ID NO: 73 - protein, 19 aa, Artificial
  Synthetic peptide
ACPLVNPLCLAPGWTCSRS

SEQ ID NO: 74 - protein, 17 aa, Artificial
  Synthetic peptide
ACPLVNPLCLEPGWTCA

SEQ ID NO: 75 - protein, 19 aa, Artificial
  Synthetic peptide
ACPLVNPLCLEPGWTCAKR

SEQ ID NO: 76 - protein, 17 aa, Artificial
  Synthetic peptide
ACPLVNPLCLHPGWSCA

SEQ ID NO: 77 - protein, 19 aa, Artificial
  Synthetic peptide
ACPLVNPLCLHPGWSCRGQ

SEQ ID NO: 78 - protein, 19 aa, Artificial
  Synthetic peptide
  Xaa (17)..(17): Xaa is HArg
ACPLVNPLCLHPGWSCXGQ

SEQ ID NO: 79 - protein, 19 aa, Artificial
  Synthetic peptide
  Xaa (14)..(14): Xaa is 2Nal
ACPLVNPLCLHPGXSCRGQ

SEQ ID NO: 80 - protein, 19 aa, Artificial
  Synthetic peptide
ACPLVNPLCLTPGWTCTNT

SEQ ID NO: 81 - protein, 17 aa, Artificial
  Synthetic peptide
ACPMVNPLCLHPGWKCA

SEQ ID NO: 82 - protein, 17 aa, Artificial
  Synthetic peptide
ACPMVNPLCLTPGWICA

SEQ ID NO: 83 - protein, 17 aa, Artificial
  Synthetic peptide
ACPMVNPLCLHPGWTCA

SEQ ID NO: 84 - protein, 19 aa, Artificial
  Synthetic peptide
  Xaa (2)..(2): Xaa is D-Asp
  Xaa (6)..(6): Xaa is Aib
  Xaa (7)..(7): Xaa is 1Nal
  Xaa (9)..(9): Xaa is Aib
  Xaa (11)..(11): Xaa is 1Nal
  Xaa (14)..(14): Xaa is tBuGly
  Xaa (16)..(16): Xaa is HArg
  Xaa (18)..(18): Xaa is D-Asp
HXVTCXXGXFXCPXNXPXC

SEQ ID NO: 85 - protein, 18 aa, Artificial
  Synthetic peptide
  Xaa (2)..(2): Xaa is HArg
  Xaa (5)..(5): Xaa is HyP
  Xaa (6)..(6): Xaa is Hse(Me)
  Xaa (15)..(15): Xaa is D-Asp
  Xaa (17)..(17): Xaa is HArg
AXDCXXVNPLCLHPXWXC

SEQ ID NO: 86 - protein, 18 aa, Artificial
  Synthetic peptide
  Xaa (2)..(2): Xaa is HArg
  Xaa (5)..(5): Xaa is HyP
  Xaa (6)..(6): Xaa is Hse(Me)
  Xaa (15)..(15): Xaa is D-Asp
AXDCXXVNPLCLHPXWTC

SEQ ID NO: 87 - protein, 18 aa, Artificial
  Synthetic peptide
  Xaa (2)..(2): Xaa is HArg
  Xaa (5)..(5): Xaa is HyP
  Xaa (15)..(15): Xaa is D-Ala
AXDCXLVNPLCLHPXWTC

SEQ ID NO: 88 - protein, 18 aa, Artificial
  Synthetic peptide
  Xaa (2)..(2): Xaa is HArg
  Xaa (15)..(15): Xaa is D-Ala
AXDCPLVNPLCLHPXWTC

SEQ ID NO: 89 - protein, 18 aa, Artificial
  Synthetic peptide
  Xaa (5)..(5): Xaa is HyP
ARDCXLVNPLCLHPGWTC

SEQ ID NO: 90 - protein, 18 aa, Artificial
  Synthetic peptide
  Xaa (13)..(13): Xaa is D-3,3-DPA
ARDCPLVNPLCLXPGWTC

SEQ ID NO: 91 - protein, 20 aa, Artificial
  Synthetic peptide
ARDCPLVNPLCLHPGWTCLH

SEQ ID NO: 92 - protein, 18 aa, Artificial
  Synthetic peptide
  Xaa (2)..(2): Xaa is HArg
  Xaa (15)..(15): Xaa is Cya
AXDCPLVNPLCLHPXWTC

SEQ ID NO: 93 - protein, 18 aa, Artificial
  Synthetic peptide
  Xaa (2)..(2): Xaa is D-Arg
  Xaa (5)..(5): Xaa is HyP
  Xaa (13)..(13): Xaa is D-3,3-DPA
  Xaa (15)..(15): Xaa is D-Asp
  Xaa (17)..(17): Xaa is HArg
AXDCXLVNPLCLXPXWXC

SEQ ID NO: 94 - protein, 17 aa, Artificial
  Synthetic peptide
ACPWGPAWCPVNRPGCA

SEQ ID NO: 95 - protein, 17 aa, Artificial
  Synthetic peptide
ACPWGPFWCPVNRPGCA

SEQ ID NO: 96 - protein, 20 aa, Artificial
  Synthetic peptide
ADVTCPWGPFWCPVNRPGCA

SEQ ID NO: 97 - protein, 15 aa, Artificial
  Synthetic peptide
CPLVNPLCLHPGWTC

SEQ ID NO: 98 - protein, 7 aa, Artificial
  Synthetic peptide
  Xaa (3)..(3): Xaa is Cit
  Xaa (5)..(5): Xaa is hPhe
EPXGXYL